European Patent Application EP 4 349 368 A1, published April 10, 2024. Title: Combination use of Immune checkpoint inhibitor and anti-C26 antibody for cancer treatment. Applicant: Y's AC Co., Ltd. The sequence listing filed with the application follows.

SEQUENCE LISTING (29 sequences)

SEQ ID NO: 1 - protein, 107 aa, Artificial Sequence
  Synthetic peptide
DILMTQSPSSLSASPGDRVTISCRASQDIRNNLNWYQQKPGQAPRLLIYYSSNLHSGVPDRFSGSGSGTDFTLTISRLEPEDFAAYYCQQSIKLPLTFGSGTKVEIK

SEQ ID NO: 2 - protein, 107 aa, Artificial Sequence
  Synthetic peptide
EIELTQSPSSLSVSLGDRVTISCSASQDIRNNLNWYQQKPGQAPRLLIYYSSNLQTGVPARFSGSGSGTDFTLTISRLEPEDVAAYYCQQSIKLPFTFGSGTKVEIK

SEQ ID NO: 3 - protein, 107 aa, Artificial Sequence
  Synthetic peptide
DIEMTQSPSSLSASAGERVTISCRASQGIRNSLNWYQQKPGQAPRLLIYYSSNLQTGVPSRFSGSGSGTDFTLTISRLQAEDFATYYCQQSNKLPFTFGSGTKVEIK

SEQ ID NO: 4 - protein, 107 aa, Artificial Sequence
  Synthetic Peptide
DILLTQSPSSLSATPGERATITCRASQGIRNNLNWYQQKPGQAPRLLIYYSSNLQSGVPSRFSGSGSGTDFTLTISRLQPEDVAAYYCQQSIKLPFTFGSGTKVEIK

SEQ ID NO: 5 - protein, 107 aa, Artificial Sequence
  Synthetic peptide
EIEMTQSPSSLSVSAGERATISCSASQDIRNSLNWYQQKPGQAPRLLIYYSSNLHTGVPARFSGSGSGTDFTLTISRLEPEDVAIYYCQQSNKLPLTFGSGTKVEIK

SEQ ID NO: 6 - protein, 107 aa, Artificial Sequence
  Syntetic peptide
EIELTQSPSSLSVSPGDRVTISCSASQGIRNSLNWYQQKPGQAPRLLIYYSSNLHTGVPARFSGSGSGTDFTLTISRLQAEDFATYYCQQSIKLPLTFGSGTKVEIK

SEQ ID NO: 7 - protein, 107 aa, Artificial Sequence
  Synthetic peptide
DILMTQSPSSLSASPGDRVTISCRASQDIRNNLNWYQQKPGQAPRLLIYYSSNLQTGVPARFSGSGSGTDFTLTISRLEPEDFAAYYCQQSIKLPLTFGSGTKVEIK

SEQ ID NO: 8 - protein, 116 aa, Artificial Sequence
  Synthetic peptide
EVQLVESGAGVKQPGGTLRLTCTASGFSLTTYGVHWVRQAPGKGLEWVGVIWGDGRTDYDAAFMSRVTISKDTSKSTVYLQMNSLRAEDTAVYYCMRNRHDWFDYWGQGTTVTVSS

SEQ ID NO: 9 - protein, 116 aa, Artificial Sequence
  Synthetic peptide
EVQLVQSGGGVKQPGETLRLTCTASGFSLTTYGVHWVRQAPGKGLEWVGVIWGDGRTDYDAAFMSRVTISKDTSKSTAYLQMNSLRAEDTAVYYCMRNRHDWFDYWGQGTTVTVSS

SEQ ID NO: 10 - protein, 116 aa, Artificial Sequence
  Synthetic peptide
EVQLVESGAGVEQPGGTLRLTCTASGFSLTTYGVHWVRQAPGKGLEWMGVIWGDGRTDYDAAFMSRVTISRDTSKSTAYLQLNSLRAEDTAVYYCVRNRHDWFDYWGQGTTVTVSS

SEQ ID NO: 11 - protein, 116 aa, Artificial Sequence
  Synthetic peptide
EVQLVESGAELVQPGGSLRLTCKASGFTLNTYGVHWVRQAPGKGLEWMGVIWGGGRTDYDASFMSRVTISKDNSKNTAYLQLNSLRAEDTAVYYCTRSRHDWFDYWGQGTTVTVSS

SEQ ID NO: 12 - protein, 116 aa, Artificial Sequence
  Synthetic peptide
EVQLVQSGGGLKQPGETLRLSCTASGYSLTTYGVHWVRQAPGKGLEWMGVIWGDGRTDYDSSFMSRVTISKDTSKSTAYLQLNSLRAEDTAVYYCTRNRHDWFDYWGQGTTVTVSS

SEQ ID NO: 13 - protein, 116 aa, Artificial Sequence
  Synthetic peptide
EVQLVQSGGGVKQPGETLRLTCTASGFSLSTYGVHWVRQAPGKGLEWVGVIWGDGRTDYDAAFMSRVTISKDTSKSTVYLQMNSLRAEDTAVYYCMRNRHDWFDYWGQGTTVTVSS

SEQ ID NO: 14 - protein, 116 aa, Artificial Sequence
  Synthetic peptide
EVQLVESGGGVKQPGETLRLTCTASGFSLSTYGVHWVRQAPGKGLEWVGVIWGDGRTDYDAAFMSRVTISKDTSKSTVYLQMNSLRAEDTAVYYCMRNRHDWFDYWGQGTTVTVSS

SEQ ID NO: 15 - protein, 116 aa, Artificial Sequence
  Synthetic peptide
  MISC_FEATURE (6)..(6): Xaa is Glu or Gln
  MISC_FEATURE (9)..(9): Xaa is Ala or Gly
  MISC_FEATURE (10)..(10): Xaa is Gly or Glu
  MISC_FEATURE (11)..(11): Xaa is Leu or Val
  MISC_FEATURE (12)..(12): Xaa is Val, Lys or Glu
  MISC_FEATURE (16)..(16): Xaa is Gly or Glu
  MISC_FEATURE (17)..(17): Xaa is Thr or Ser
  MISC_FEATURE (21)..(21): Xaa is Thr or Ser
  MISC_FEATURE (23)..(23): Xaa is Thr or Lys
  MISC_FEATURE (27)..(27): Xaa is Phe or Tyr
  MISC_FEATURE (28)..(28): Xaa is Ser or Thr
  MISC_FEATURE (30)..(30): Xaa is Thr, Asn or Ser
  MISC_FEATURE (48)..(48): Xaa is Val or Met
  MISC_FEATURE (54)..(54): Xaa is Gly or Asp
  MISC_FEATURE (61)..(61): Xaa is Ala or Ser
  MISC_FEATURE (62)..(62): Xaa is Ala or Ser
  MISC_FEATURE (71)..(71): Xaa is Lys or Arg
  MISC_FEATURE (73)..(73): Xaa is Asn or Thr
  MISC_FEATURE (76)..(76): Xaa is Ser or Asn
  MISC_FEATURE (78)..(78): Xaa is Val or Ala
  MISC_FEATURE (82)..(82): Xaa is Met or Leu
  MISC_FEATURE (96)..(96): Xaa is Val, Met or Thr
  misc_feature (98)..(98): Xaa can be any naturally occurring amino acid
EVQLVXSGXXXXQPGXXARLXCXASGXXLXTYGVHWVRQAPGKGLEWXGVIWGXGRTDYDXXFMSRVTISXDXSKXTXYLQXNSLRAEDTAVYYCXRXRHDWFDYWGQGTTVTVSS

SEQ ID NO: 16 - protein, 107 aa, Artificial Sequence
  Synthetic peptide
  MISC_FEATURE (1)..(1): Xaa is Asp or Glu
  MISC_FEATURE (3)..(3): Xaa is Leu or Glu
  MISC_FEATURE (4)..(4): Xaa is Met or Leu
  MISC_FEATURE (13)..(13): Xaa is Ala or Val
  MISC_FEATURE (14)..(14): Xaa is Ser or Thr
  MISC_FEATURE (15)..(15): Xaa is Leu, Pro or Ala
  MISC_FEATURE (17)..(17): Xaa is Asp or Glu
  MISC_FEATURE (19)..(19): Xaa is Val or Ala
  MISC_FEATURE (22)..(22): Xaa is Thr or Ser
  MISC_FEATURE (24)..(24): Xaa is Ser or Arg
  MISC_FEATURE (28)..(28): Xaa is Gly or Asp
  MISC_FEATURE (32)..(32): Xaa is Ser or Asn
  MISC_FEATURE (55)..(55): Xaa is His or Gln
  MISC_FEATURE (56)..(56): Xaa is Ser or Thr
  MISC_FEATURE (60)..(60): Xaa is Ser, Asp or Ala
  MISC_FEATURE (79)..(79): Xaa is Glu or Gln
  MISC_FEATURE (80)..(80): Xaa is Pro or Ala
  MISC_FEATURE (83)..(83): Xaa is Phe or Val
  MISC_FEATURE (85)..(85): Xaa is Thr, Ala or Ile
  MISC_FEATURE (92)..(92): Xaa is Ile or Asn
  MISC_FEATURE (96)..(96): Xaa is Phe or Leu
XIXXTQSPSSLSXXXGXRXTIXCXASQXIRNXLNWYQQKPGQAPRLLIYYSSNLXXGVPXRFSGSGSGTDFTLTISRLXXEDXAXYYCQQSXKLPXTFGSGTKVEIK

SEQ ID NO: 17 - protein, 465 aa, Artificial Sequence
  Synthetic pepitde
MEWSWVFLFFLSVTTGVHSEVQLVESGAGVKQPGGTLRLTCTASGFSLTTYGVHWVRQAPGKGLEWVGVIWGDGRTDYDAAFMSRVTISKDTSKSTVYLQMNSLRAEDTAVYYCMRNRHDWFDYWGQGTTVTVSSASTKGPSVFPLAPSSKSTSGGTAALGCLVKDYFPEPVTVSWNSGALTSGVHTFPAVLQSSGLYSLSSVVTVPSSSLGTQTYICNVNHKPSNTKVDKKVEPKSCDKTHTCPPCPAPELLGGPSVFLFPPKPKDTLMISRTPEVTCVVVDVSHEDPEVKFNWYVDGVEVHNAKTKPREEQYNSTYRVVSVLTVLHQDWLNGKEYKCKVSNKALPAPIEKTISKAKGQPREPQVYTLPPSRDELTKNQVSLTCLVKGFYPSDIAVEWESNGQPENNYKTTPPVLDSDGSFFLYSKLTVDKSRWQQGNVFSCSVMHEALHNHYTQKSLSLSPGK

SEQ ID NO: 18 - protein, 234 aa, Artificial Sequence
  Synthetic peptide
MSVPTQVLGLLLLWLTDARCDILLTQSPSSLSATPGERATITCRASQGIRNNLNWYQQKPGQAPRLLIYYSSNLQSGVPSRFSGSGSGTDFTLTISRLQPEDVAAYYCQQSIKLPFTFGSGTKVEIKRTVAAPSVFIFPPSDEQLKSGTASVVCLLNNFYPREAKVQWKVDNALQSGNSQESVTEQDSKDSTYSLSSTLTLSKADYEKHKVYACEVTHQGLSSPVTKSFNRGEC

SEQ ID NO: 19 - protein, 13 aa, Artificial Sequence
  Synthetic peptide
YSLRWISDHEYLY

SEQ ID NO: 20 - protein, 13 aa, Artificial Sequence
  Synthetic peptide
LEYNYVKQWRHSY

SEQ ID NO: 21 - protein, 13 aa, Artificial Sequence
  Synthetic peptide
TWSPVGHKLAYVW

SEQ ID NO: 22 - protein, 13 aa, Artificial Sequence
  Synthetic peptide
LWWSPNGTFLAYA

SEQ ID NO: 23 - protein, 13 aa, Artificial Sequence
  Synthetic peptide
RISLQWLRRIQNY

SEQ ID NO: 24 - protein, 13 aa, Artificial Sequence
  Synthetic peptide
YVKQWRHSYTASY

SEQ ID NO: 25 - protein, 13 aa, Artificial Sequence
  Synthetic peptide
EEEVFSAYSALWW

SEQ ID NO: 26 - protein, 13 aa, Artificial Sequence
  Synthetic peptide
DYSISPDGQFILL

SEQ ID NO: 27 - protein, 13 aa, Artificial Sequence
  Synthetic peptide
SISPDGQFILLEY

SEQ ID NO: 28 - protein, 13 aa, Artificial Sequence
  Synthetic peptide
IYVKIEPNLPSYR

SEQ ID NO: 29 - protein, 15 aa, Artificial Sequence
  Synthetic peptide
GGGGSGGGGSGGGGS